European Patent Application EP 4 677 998 A1, published January 14, 2026. Title: A method of producing a plant with an increased density of glandular trichomes and/or an increased production of metabolites. Applicant: Institut national de recherche pour l'agriculture, l'alimentation et l'environnement. Application EP. The sequence listing filed with the application follows.

SEQUENCE LISTING (59 sequences)

SEQ ID NO: 1 - protein, 725 aa, Salvia sclarea
MFQPNMFDSHHHLLDMAHKTPENEMDLIRDEEYESKSGTDIMEAPSGDDQDPNQRPKKKRYHRHTQHQIQEMESFFNECPHPDDKQRKELGRRLGLEPLQVKFWFQNKRTQMKAQHERHENTQLRNENEKLRAENIRYKEALSNATCPNCGGPAAIGEMSFDEQHLRIENARLREEIDRISGIAAKYVGKPMLSYPHLSPGASRSLDLGVGNFGSQTGIGGEVYGAGDLLRSVSGPTDADKPVIIELAVAAMEELIRMAQSGDPLWIPSTENGAEILSEEEYGRTFPRGIGPKPLGLKSEASRESAVVIMNHINLVEILMDVNQWSNVFASIVSRSVTLEVLSTGVAGNYNGALQVMTAEFQVPSPLVPTRENYFVRYCKQHTDGTWAVVDVSLDNLRPTSISRCRRRPSGCLIQELPNGYSKVTWVEHVEVDDRAVHSIYKPLVNSGLAFGAKRWVATLDRQCERLASVMANNISAGDVGVISTPEGRKSMLKLAERMVMSFCTGVGASTAHTWTTLSGSGADDVRVMTRKSMDDPGRPPGIVLSAATSFWLPVPPKRVFDFLRDENSRSEWDILSNGGLVQEMAHIANGRDPGNSVSLLRVNSANSSQSNMLILQESSTDATGSYVIYAPVDIHAMNIVLSGGDPDYVALLPSGFAILPDGPTNEAPGVPEVGSGGSLLTVAFQILVDSVPTAKLSLGSVATVNSLIKCTVERIKGAVLCDTA

SEQ ID NO: 2 - protein, 774 aa, Cannabis sativa
MFQPNMFETTHHHHHHLMDISHNKSISESDQLGLGANMRDDDLETKSGTELIMEADPSGDDELDPTQKSKRKRYHRHTQRQIQEMEAFFKECPHPDDKQRKELSRELGLEPLQVKFWFQNKRTQMKAQHERHENSILKAENDKLRAENNRYKEALSNATCPNCGGPAALGEMSFDEQHLRIENARLREEIDRISGIAAKYAGKPLSSFSHLSSHASRTLDISGVGNFGSQSGFVGEMFGATGDLLRSVSVPTEADKPIIVELAVAAMEELIRMAQAGDPLWIPAHHDNNSISGGNNSTEILNEDEYLRTFPRGIGPKPLGMKSEASRETNVVIMNHTNLVEILMDVNQWSTIFCGIVSRAMTLDILSTGVAGNYNGALQVMTAEFQVPSPLVPTRENYFVRYCKQHGDGTWAVVDVSLDNLRPSPISRSRRRPSGCLIQELPNGYSKVTWVEHVEVDDRAVHNIYKPLVNSGIAFGAKRWVATLDRQCERLASSMASNIPAGDLCVITSPDGRKSMLKLAERMVMSFCVGVGASTAHAWTTLSATGSDDVRVMTRKSMDDPGRPPGIVLSAATSFWLPVPPKRVFDFLRDENSRSEWDILSNGGLVQEMAHIANGRDPGNCVSLLRVNSANSSQSNMLILQESCTDSTGSYVIYAPVDIVAMNVVLSGGDPDYVALLPSGFAILPDGPANNNNNINNNNNSHNSGIINNNGPAGSGIVEVGSGGSLLTVAFQILVDSVPTAKLSLGSVATVNNLIKCTVERIRAAVTSENVQGA

SEQ ID NO: 3 - protein, 725 aa, Artemisia annua
MFQPNMFESHHHILDISCKTSENQLDMLRDEDYESKSGTDIMEAPSGDEQDPNQRPNKKKRYHRHTQHQIQEMESFFKECPHPDDKQRKELGRRLTLEPLQVKFWFQNKRTQMKAQHERHENTQLRNENEKLRSENIRYKEALANATCPNCGGPAAIGEMSFDEQQLRIENTRLHEEIDRISGIAAKYVGKPVLSYPNMPSHGPTRSLDLGVPNFGPQQGMVGDMFGANDLLRSVSGPTEADKPIIIELAVAAMEELIRMAQAGDPLWVQNSDTSSEVLSEEEYMRTFPRGIGPKPLGLISEASRESAVVIMNHITLVEILMDVNQWSNVFSGIVSRAMTLEVLSTGVAGNYNGALQVMTAEYQVPSPLVPTRENYFVRYCKQHSDGTWAVVDVSLDNLRTSSISRCRRRPSGCLIQELPNGYSKVTWVEHVEVDDRSVHEIYRSLVTSGLGFGAKRWVKTLERQCERLASVMANNIPAGDVGVITTPEGRKSMLKLAERMVLSFCSGVGASTAHTWTTLSGSGADDVRVMTRKSMDDPGRPPGIVLSAATSFWIPIQPKRVFDFLRDENSRSEWDILSNGGLVQEMAHIANGRDPGNCVSLLRVNSANSSQSNMLILQESSSDATGSYVIYAPVDIVAMNVVLSGGDPDYVALLPSGFAILPDGPGQQEGGNPEVGTGGSLLTVAFQILVDSIPTAKLSLGSVATVNSLIKCTVERIKAAVASP

SEQ ID NO: 4 - protein, 727 aa, Salvia splendens
MFQPNMFDSHHHLLDMAHKTPENEMDLIRDDEYGSKSGTDIMEAPSGDDQDPNQRPKKKRYHRHTQHQIQEMESFFNECPHPDDKQRKELGRRLGLEPLQVKFWFQNKRTQMKAQHERHENTQLRNENDKLRADNIRYKEALTNATCPSCGGPAAIGEMSFDEQHLRIENARLREEIDRISGIASKYVGKPMLSYPHLSPGGGASRSLDLGVGNFGGQSGIGGEVFGAADLLRSVSGPTEADKPVIIELAVAAMEELIRMAQAGEPLWIPSINNGAEMLSEEDYGTTFPRGIGPKPLGLISEASRELAVVIMNHINLVEILMDVNQWSSMFASIVSRAVTVEVLSTGVAGNHNGALQVMTAEFQVPSPLVPTRENYFVRYCKQHTDGTWAVVDVSLDNLRPSSISRCRRRPSGCLIQELPNGYSKVTWVEHVEIDDRAVHSIYKPLVNSGLAFGAKRWVATLDRQCERLASVMANNISAGDVGVISSPEGRKSMLKLAERMVMSFCSGVGASTAHTWTTLSGSGADDVRVMTRKSMDDPGRPPGIVLSAATSFWLPVSPKRVFDFLRDENSRSEWDILSNGGLVQEMAHIANGRDPGNSVSLLRVNSANSSQSNMLILQESSTDATGSYVIYAPVDIHAMNVVLSGGDPDYVALLPSGFAILPDGPSNEAGGVEVGSGGSLLTVAFQILVDSVPTAKLSLASVTTVNNLIKCTVERIKGAVLCDTAV

SEQ ID NO: 5 - protein, 723 aa, Salvia hispanica
MFQPNMFDGHHHLLEMAQKTPENEMDPIRDEEYESRSGTDIMEVPSGDEQDPNQRPKKKRYHRHTQLQIQEMESFFNECPHPDDKQRKELGRRLGLEPLQVKFWFQNKRTQMKAHHERHENSQLRNDNEKLRAENIRYKEALGNATCPNCGGPAAIGEMSFDEQHLRIENARLREEIDRISGIAAKYVGKPMLPTYPPIAPGPSRSLDLGVGSFAADSGDVFGAGDILRSVSGPTEADKPVIIELAVAAMEELVRMAQAGEPLWLQTTENGVELFCEEEYARTFPRGIGPKPLGLKSEASRESAVVIMNHISLVEILMDVNQWSNVFASIVSRSATLEVLSTGVAGNYNGAFQVMTAEFQVPSPLVPTRENYFVRYCKQHHDGTWAVVDVSLDNLRPASISRCRRRPSGCLIQELPNGYSKVTWIEHVEVDDRAVHSIYKALVNSGLAFGAKRWVATLDRQCERLASVMANNISAGDVGVISSPEGRKSMLKLAERMVMSFCTGVGASTAHTWTTLSGIGADDVRVMTRKSMDDPGRPPGIVLSAATSFWIPVPPKRVFDFLRNENARNEWDILSNGGLVQEMAHIANGRDPGNSVSLLRVNSANSSQSNMLILQESSTDETGSYVIYAPVDIHAMNVVLSGGDPDYVALLPSGFAILPDGPSEEDGGIPEGVSGGSLLTVAFQILVDSVPTAKLSLGSVATVNSLIKCTVERIKAAVVCDAA

SEQ ID NO: 6 - protein, 712 aa, Perilla frutescens
MGNKSPENEMELIRDDDYESKSGTDNMEAPSGDDQDPNDRPKKKRYHRHTQNQIQEMESFFKECPHPDDKQRKELGRRLGLEPLQVKFWFQNKRTQMKSQHERHENTQLRNDNEKLRAENIRYKEALSNATCPSCGGPAAIGEMSFDEQHLRIENSRLREEIDRISGIAAKYVGKPMLSAYPPLPPGASRSLDLGVGSFGANAGMAGEIYGAAADLLRSVSGPSDADKPVIIELAVAAMEELLRMGQTGEPLWIPSSDSSGEVLSDDEYVRTFPRGIGPKPLGLRSEASRESAVVIMNHINLVEILMDTTQWSSVFSSIVSRAMTLEVLSTGVAGNYNGALQVMTAEFQVPSPLVPTREIYFVRYCKQHGDGTWAVVDVSLDNLRPSNISKCRRRPSGCLIQELPNGYSKVTWVEHVEVDDRAVHSIYKPLVNSGLAFGARRWVAILDRQCERLASVMANNISSGDVGVISSPKGRKSMLKLAERMVMSFCTGVGASTAHTWTTLSGSGADDVRVMTRKSMDDPGRPPGIVLSAATSFWLPVPPKRVFDFLRDENSRNEWDILSNGGLVQEMAHIANGRDPGNSVSLLRVNSANSSQSNMLILQESCTDTTGSYVIYAPVDIIAMNVVLSGGDPDYVALLPSGFAILPDGAIDQTGGIPEVGSGGSLLTVAFQILVDSVPTAKLSLGSVATVNSLIKCTVERIKGAVLHDGA

SEQ ID NO: 7 - protein, 725 aa, Thymus quinquecostatus
MFQPNMFDSHHHLLDMGHKTPENEMDLIRDDEYESKSGTDIMEAASGDEQDPNQRPKKKRYHRHTQHQIQEMESFFNECPHPDDKQRKELGRRLGLEPLQVKFWFQNKRTQMKAQHERHENTQLRNENEKLRAENVRYKEALSNATCPNCGGPAAIGEMSFDEQHLRIENARLREEIDRISGIAAKYVGKPMLSYPHLAPGASRSSLDLGVGNFGPQAGITGEVFGAADLLRSVSGPTDADKPVIIELAVAAMEELIRMAQAGEPLWIPSTENLGEVLVEEEYGRTFPRGIGPKPIGLKSEASRQTSVVIMNHINLVEILMDVNQWSNVFASIVSRAVTLEVLSTGVAGNYNGALQVMTAEFQVPSPLVPTRENYFVRYCKQHTDGSWAVVDVSLDNLRPTSISKCRRRPSGCVIQELPNGYSKVTWIEHVEVDDRAVHSIYKPLVNAGLAFGAKRWVATLDRQCERLASVMANNISAGEIGVISSPEGRKSMLKLAERMVMSFCTGVGASTAHTWTTLSGSGADDVRVMTRKSMDDPGRPPGIVLSAATSFWLPVPPKRVFDFLRDENSRSEWDILSNGGLVQEMAHIANGRDPGNSVSLLRVNSANSSQSNMLILQESSTDATGSYVIYAPVDIHAMNIVLGGGDPDYVALLPSGFAILPDGPHTEGGGIPEVGSGGSLLTVAFQILVDSVPTAKLSLGSVATVNSLIKCTVERIKGAVLCET

SEQ ID NO: 8 - protein, 727 aa, Mentha longifolia
MFQPNMFDSHHHLLDMGHKTPENDMDLIRDDEYESKSGTDIMENASGDEQDPNQRPKKKRYHRHTQHQIQEMESFFNECPHPDDKQRKELGRRLGLEPLQVKFWFQNKRTQMKAQHERHENTQLRNENEKLRAENIRYKEALSNATCPNCGGPAAIGEMSFDEQHLRIENARLREEIDRISGIAAKYVGKPMLSYPHLAPGASRSSLDLGVGNFGPQTGITGEVFGAADLLRSVSGPTDADKPVIIELAVAAMEELIRMAQTGEPLWIPSTENSSGEVLSEEEYGRTFPRGIGPKPLGLKSEASRETSVVIMNHINLVEILMDVNQWSNVFASIVSRAVTLEVLSTGVAGNYNGALQVMTAEFQVPSPLVPTRENYFVRYCKQHTDGTWAVVDVSLDNLRPTSISKCRRRPSGCLIQELPNGYSKVTWIEHVEVDDRTVHSIYKPLVNAGLAFGARRWVATLDRQCERLASVMANNISAGDVGVISSPEGRKSMLKLAERMVMSFCTGVGASTAHTWTTLSGSGADDVRVMTRKSMDDPGRPPGIVLSAATSFWLPVPPKRVFDFLRDENSRSEWDILSNGGLVQEMAHIANGRDPGNSVSLLRVNSANSSQSNMLILQESSTDATGSYVIYAPVDIHAMNVVLSGGDPDYVALLPSGFAILPDGPHSEGGGIPEVGSGGSLLTVAFQILVDSVPTAKLSLGSVATVNSLIKCTVERIKGAVLCETA

SEQ ID NO: 9 - protein, 712 aa, Solanum lycopersicum
MFQHNMFDSHNFLLDMTRKTPENELDLIRDDEFETKSGADIMEGGASGDDQDPNKRPKKKQYHRHTQHQIQELESFFKECPHPDDKQRKDLGKRLGLEPLQVKFWFQNKRTQMKSQHERHENTQLRNENDKLRAENIRYKEALTTATCPNCGGPAAIGEMSFDEQHLRIENARLREEIDRISGIAAKYVGKPMLNYPQLPSLGGNILGEMFTTTTSAGDLLRSISGPTDADKPIVIELAVAAMEELIRLAQTDEPLWMNQNSDNNDLILNEEEYARTFPRGIGPKSLGLKSEASRESAVVIIDYLHLVEILMDVSQWTNFFTGIVSKSTILEVLSTGVAGNYNGALQVMTAEFQVPSPLVPTRENYFVRYCKQHGDGTWAVVDVSLENLRSTSVSRCRRRPSGCVIQELPNGYSKVTWIEHVEVDDRAVNNIYRPLVDSGLAFGAKRWVATLERQCERLASVMASNIPTGDVITSPEGRKSMLKLAERMVMSFCAGVGASTAHTWTTLSGSGADDVRVMTRKSIDDPGRPPGIVLSAATSFWMPVPTKRVFDFLRDENSRNEWDILSNGGLVQEMAHIANGRDSGNSVSLLRVNSGNSSQNNMLILQESCLDITGSYVIYAPVDIAAMNVVLSGGDPDYVALLPSGFAILPDGSSNAENSNIAGGSLLTVAFQILVDSVPTAKLSLGSVATVNSLIKCTVERIKASITCENA

SEQ ID NO: 10 - protein, 727 aa, Solanum tuberosum
MFQPNMFESHHHLLDMSHKSPENDLDLLRDNDEFESKSMADIMENNPSGDDQEADPNQRPNKKKRYHRHTQLQIQEMESFFKECPHPDDKQRKELGKRLGLEPLQVKFWFQNKRTQMKAQHERHENSELRAENEKLRADNIRYKEALGNATCPNCGGPASIGEMSFDEQHLRIENARLREEIDRISGIAAKYVGKPMLTYPNLPIGPTRSLDIGVGSFGPQTGLVGEMYSAGDLLRSVSGPIDADKPMIIELAVAAMEELVRMAQTGEPLWITGPGPDNSMETLCEEEYVRTFPRGIGPKSLGLTTEASRESAVVIMNHINLVEILMDVNQWTNVFAGLVSRALTLDVLSTGVAGNYNGALQVMTAEFQVPSPLVPTRENYFVRYCKHHTDGTWAVVDVSLDNLRPSSVSHGRRRPSGCLIQELPNGYSKVTWIEHVEVDDRGVHNIYRPLVNSGLAFGAKRWVATLDRQCERLASAMANNIPTGDIGVITSPEGRKSMLKLAERLVMSFCAGVGASTAHTWTTLSGSGADDVRVMTRKSIDDPGRPPGIVLSAATSFWLPVPPKRVFDFLRDENSRSEWDILSNGGLVQEMAHIANGRDPGNCVSLLRVNSGNSSQSNMLILQESSTDSTGSYVIYAPVDIVAMNVVLSGGDPDYVALLPSGFAILPDGGGGIDVGTRGSLLTVAFQILVDSVPTAKLSLGSVATVNSLIKCTVERIKTAVACDNA

SEQ ID NO: 11 - protein, 728 aa, Capsicum annuum
MFQPNMFESHHHLLDMSHNKSPENDLDLIRDDEFESKSMADIMENNPCGDDNEDPNQRPNKKKRYHRHTQIQIQEMESFFKECPHPDDKQRKELGKKLGLEPLQVKFWFQNKRTQMKAQHERHENSELRAENEKLRAENIRYKEALGNASCPNCGGPASIGEMSFDEQHLRIENARLREEIDRISGIAAKYVGKPMLTYPNLSTTGPLDLGVGNFGPQTGLVGEIYNASDLLRSVSGPIDADKPIIIELAVAAMEELIRMAQTGEPLWIKTLDNSSETLSEEEYFRTFPQGIGPKPLGLTSEASRESAVVIMNHINLVEILMDVNQWTSVFAGLVSRSLTLEVLSTGVAGNYNGALQVMTAEFQVPSPLVPTRENYFVRYCKHHADGTWAVVDVSLDHLRPTAVSRDRRRPSGCLIQELPNGYSKVTWIEHVEVDDRSAHNIYRPLVNSGLAFGAKRWVATLDRQCERLASAMAINIPTGEVGVITSPDGRKSMLKLAERMVMSFCAGVGASTAHTWTTLSGSGADDVRVMTRKSIDDPGRPPGIVLSAATSFWLPVSPKRVFDFLRDENSRNEWDILSNGGLVQEMAHIANGRDPGNCVSLLRVNSGNSSQSNMLILQESSTDSTGSYVIYAPVDIVAMNVVLSGGDPDYVALLPSGFAILPDGGGGINTTCTSGSLLTVAFQILVDSIPTAKLSLGSVATVNSLLKCTVERIKNALACDTMPDGKI

SEQ ID NO: 12 - protein, 723 aa, Cucumis melo
MFQPSIMDAHLLPLDIPQNTSESDLARIRDDDFDSATKSGSDNNHELVSGDDQDPRPKKKRYHRHTQHQIQEMEAFFKECPHPDDKQRKELSRELGLEPLQVKFWFQNKRTQMKNQHERHENTQLRTENEKLRADNMRYREALSNASCPNCGGPTAIGEMSFDEHHLRLENARLREEIDRISAIAAKYVGKPVVNYPLLSPPVPSRPLELGMANFGPQPGLGGGDIYGSASDLIRSISAPTEADKPMIIELAVAAMEELTRMAQMGEPLWMTTLDGSTHMLNEDEYLRTFPRGIGPKPSGFKCEASRESAVVIMNHINLVEILMDVNQWSTLFSGIVSRAMTLEVLSTGVAGNYNGALQVMTSEFQVPSPLVPTRESYFVRYCKQHGDGTWAVVDVSLDDLRPTPGVRCRRRPSGCLIQEMPNGYSKVTWVEHVEVDDRGVHNLYKQLVSSGQAFGAKRWVTTLDRQCERLASAMATNIPTGDVGVITNQEGRKSMLKLAERMVISFCAGVSASTTHTWTTLSGTGADDVRVMTRKSIDDPGRPHGIVLSAATSFWLPVPPKRIFDFLRDENSRSEWDILSNGGVVQEMAHIANGRDTGNCVSLLRVNSANSSQSNMLILQESCTDPTASFVIYAPVDVVAMNLVLNGGDPDYVALLPSGFAILPDGGGGEGVSGGSLLTVAFQILVDSVPTAKLSLGSVATVNNLIACTVERIKASLSCENA

SEQ ID NO: 13 - protein, 723 aa, Cucumis sativus
MFQPSIMDAHLLPLDIPQNTSESDLARIRDDDFDSATKSGSDNNHELVSGDDQDPRPKKKRYHRHTQHQIQEMEAFFKECPHPDDKQRKELSRELGLEPLQVKFWFQNKRTQMKNQHERHENTQLRTENEKLRADNMRYREALSNASCPNCGGPTAIGEMSFDEHHLRLENARLREEIDRISAIAAKYVGKPVVNYPLLSPSVPSRPLELGMANFGPQPGLGGGDIYGSASDLIRSISAPTEADKPMIIELAVAAMEELTRMAQMGEPLWMTTLDGSTHMLNEDEYLRTFPRGIGPKPSGFKCEASRESAVVIMNHINLVEILMDVNQWSTLFSGIVSRAMTLEVLSTGVAGNYNGALQVMTSEFQVPSPLVPTRESYYVRYCKQHGDGTWVVVDVSLDDLRPTPGVRCRRRPSGCLIQEMPNGYSKVTWVEHVEVDDRGVHNLYKQLVSSGQAFGAKRWVTTLDRQCERLASAMATNIPTGDVGVITNQEGRKSMLKLAERMVISFCAGVSASTTHTWTTLSGTGADDVRVMTRKSIDDPGRPHGIVLSAATSFWLPVPPKRIFDFLRDENSRSEWDILSNGGVVQEMAHIANGRDTGNCVSLLRVNSANSSQSNMLILQESCTDPTASFVIYAPVDVVAMNLVLNGGDPDYVALLPSGFAILPDGGGGEGVSGGSLLTVAFQILVDSVPTAKLSLGSVATVNNLIACTVERIKASLSCENA

SEQ ID NO: 14 - protein, 725 aa, Gossypium hirsutum
MFSPNLFESPHMFDMSHKTSESELMGKIRDDDYEIKSVNETMDAPSGDDQDPDQRPKKKRYHRHTQRQIQEMEAFFKECPHPDDKQRKELGRELGLEPLQVKFWFQNKRTQMKAQHERHENAILKAENEKLRAENNRYKEALSNATCPSCGGPAALGEMSFDEQHLRIENARLREEIDRISGIAAKYVGKPLSSLPHLSSHLHSRSADLGASNFGNQSGFVGEMDRSGDLLRSVSGPTEADKPMIVELAVAAMEELIRMAQSGEPLWVPGDNSTDVLNEDEYLRTFPRGIGPKPLGLRSEASRESAVVIMNHVNLVEILMDVNQWSSVFCGIVSRAMTLEVLSTGVAGNYNGALQVMTAEFQVPSPLVPTRENYFARYCKQHIDGTWAVVDVSLDNLRPNPMSKCRRRPSGCLIQELPNGYSKVIWVEHVEVDDRAVHNIYRPVVNSGLAFGAKRWVATLDRQCERLASSMASNIPAGDLCVITSPEGRKSMLKLAERMVTSFCTGVGASTAHAWTTLSATGSDDVRVMTRKSMDDPGRPPGIVLSAATSFWIQVPPKRVFDFLRDENSRSEWDILSNGGLVQEMAHIANGRDPGNCVSLLRVNSANSSQSNMLILQESCTDAKGSYVIYAPVNIVAMNIVLSGGDPDYVALLPSGFAILPDGPGVNGGGILEIGSGGSLLTVAFQILVDSVPTAKLSLGSVATVNSLIKCTVERIKAAVKCNNA

SEQ ID NO: 15 - protein, 730 aa, Nicotiana tabacum
MFQPNMFESHHHLLDMSHKSPENELDFIRDDEFDTKSGTDIMENPSGDDQDPNQRPNKKKRYHRHTQLQIQEMESFFKECPHPDDKQRKELGKKLVLEPLQVKFWFQNKRTQMKAQHERHENSQLRNENEKLRAENIRYKEALGNATCPNCGGPAAIGEMSFDEQHLRIENARLREEIDRISGIAAKYVGKPMLTYPNLPSTGSTRSLDLGVSSFGPQTGLVGEMYSASDLLRSVSGPTDADKPIIIELAVAAMEELIRMAQTGEPLWILSPDNSTETLCVEEYMRTFPRGIGPQPLGLKSEASRESAVVIMNHINLVEILMDVNQWTSVFAGLVSRAVTLEVLSTGVAGNYNGALQVMTAEFQVPSPLVPTRENYFVRYCKHHADGTWAVVDVSLDNLRPTSTSRCRRRPSGCLIQELPNGYSKVTWIEHIEVDDRAVHNIYRPLVNSGLAFGAKRWVATLDRQCERLASAMANNIPTGDIGVITSPEGRRSMLKLAERMVMSFCAGVGASTAHTWTTLSGSGADDVRVMTRKSIDDPGRPPGIVLSAATSFWLPVPPKRVFDFLRDENSRSEWDILSNGGLVQEMAHIANGRDPGNCVSLLRVNSGNSSQSNMLILQESSTDSTGSYVIYAPVDIVAMNVVLSGGDPDYVALLPSGFAILPDGSTSSHCGGNNVVEVGNGGSLLTVAFQILVDSVPTAKLSLGSVATVNSLIKCTVERIKTAVVCDNA

SEQ ID NO: 16 - protein, 233 aa, Salvia sclarea
TDADKPVIIELAVAAMEELIRMAQSGDPLWIPSTENGAEILSEEEYGRTFPRGIGPKPLGLKSEASRESAVVIMNHINLVEILMDVNQWSNVFASIVSRSVTLEVLSTGVAGNYNGALQVMTAEFQVPSPLVPTRENYFVRYCKQHTDGTWAVVDVSLDNLRPTSISRCRRRPSGCLIQELPNGYSKVTWVEHVEVDDRAVHSIYKPLVNSGLAFGAKRWVATLDRQCERLAS

SEQ ID NO: 17 - protein, 242 aa, Cannabis sativa
TEADKPIIVELAVAAMEELIRMAQAGDPLWIPAHHDNNSISGGNNSTEILNEDEYLRTFPRGIGPKPLGMKSEASRETNVVIMNHTNLVEILMDVNQWSTIFCGIVSRAMTLDILSTGVAGNYNGALQVMTAEFQVPSPLVPTRENYFVRYCKQHGDGTWAVVDVSLDNLRPSPISRSRRRPSGCLIQELPNGYSKVTWVEHVEVDDRAVHNIYKPLVNSGIAFGAKRWVATLDRQCERLAS

SEQ ID NO: 18 - protein, 233 aa, Artemisia annua
TEADKPIIIELAVAAMEELIRMAQAGDPLWVQNSDTSSEVLSEEEYMRTFPRGIGPKPLGLISEASRESAVVIMNHITLVEILMDVNQWSNVFSGIVSRAMTLEVLSTGVAGNYNGALQVMTAEYQVPSPLVPTRENYFVRYCKQHSDGTWAVVDVSLDNLRTSSISRCRRRPSGCLIQELPNGYSKVTWVEHVEVDDRSVHEIYRSLVTSGLGFGAKRWVKTLERQCERLAS

SEQ ID NO: 19 - protein, 233 aa, Salvia splendens
TEADKPVIIELAVAAMEELIRMAQAGEPLWIPSINNGAEMLSEEDYGTTFPRGIGPKPLGLISEASRELAVVIMNHINLVEILMDVNQWSSMFASIVSRAVTVEVLSTGVAGNHNGALQVMTAEFQVPSPLVPTRENYFVRYCKQHTDGTWAVVDVSLDNLRPSSISRCRRRPSGCLIQELPNGYSKVTWVEHVEIDDRAVHSIYKPLVNSGLAFGAKRWVATLDRQCERLAS

SEQ ID NO: 20 - protein, 233 aa, Salvia hispanica
TEADKPVIIELAVAAMEELVRMAQAGEPLWLQTTENGVELFCEEEYARTFPRGIGPKPLGLKSEASRESAVVIMNHISLVEILMDVNQWSNVFASIVSRSATLEVLSTGVAGNYNGAFQVMTAEFQVPSPLVPTRENYFVRYCKQHHDGTWAVVDVSLDNLRPASISRCRRRPSGCLIQELPNGYSKVTWIEHVEVDDRAVHSIYKALVNSGLAFGAKRWVATLDRQCERLAS

SEQ ID NO: 21 - protein, 233 aa, Perilla frutescens
SDADKPVIIELAVAAMEELLRMGQTGEPLWIPSSDSSGEVLSDDEYVRTFPRGIGPKPLGLRSEASRESAVVIMNHINLVEILMDTTQWSSVFSSIVSRAMTLEVLSTGVAGNYNGALQVMTAEFQVPSPLVPTREIYFVRYCKQHGDGTWAVVDVSLDNLRPSNISKCRRRPSGCLIQELPNGYSKVTWVEHVEVDDRAVHSIYKPLVNSGLAFGARRWVAILDRQCERLAS

SEQ ID NO: 22 - protein, 233 aa, Thymus quinquecostatus
TDADKPVIIELAVAAMEELIRMAQAGEPLWIPSTENLGEVLVEEEYGRTFPRGIGPKPIGLKSEASRQTSVVIMNHINLVEILMDVNQWSNVFASIVSRAVTLEVLSTGVAGNYNGALQVMTAEFQVPSPLVPTRENYFVRYCKQHTDGSWAVVDVSLDNLRPTSISKCRRRPSGCVIQELPNGYSKVTWIEHVEVDDRAVHSIYKPLVNAGLAFGAKRWVATLDRQCERLAS

SEQ ID NO: 23 - protein, 234 aa, Mentha longifolia
TDADKPVIIELAVAAMEELIRMAQTGEPLWIPSTENSSGEVLSEEEYGRTFPRGIGPKPLGLKSEASRETSVVIMNHINLVEILMDVNQWSNVFASIVSRAVTLEVLSTGVAGNYNGALQVMTAEFQVPSPLVPTRENYFVRYCKQHTDGTWAVVDVSLDNLRPTSISKCRRRPSGCLIQELPNGYSKVTWIEHVEVDDRTVHSIYKPLVNAGLAFGARRWVATLDRQCERLAS

SEQ ID NO: 24 - protein, 234 aa, Solanum lycopersicum
TDADKPIVIELAVAAMEELIRLAQTDEPLWMNQNSDNNDLILNEEEYARTFPRGIGPKSLGLKSEASRESAVVIIDYLHLVEILMDVSQWTNFFTGIVSKSTILEVLSTGVAGNYNGALQVMTAEFQVPSPLVPTRENYFVRYCKQHGDGTWAVVDVSLENLRSTSVSRCRRRPSGCVIQELPNGYSKVTWIEHVEVDDRAVNNIYRPLVDSGLAFGAKRWVATLERQCERLAS

SEQ ID NO: 25 - protein, 235 aa, Solanum tuberosum
IDADKPMIIELAVAAMEELVRMAQTGEPLWITGPGPDNSMETLCEEEYVRTFPRGIGPKSLGLTTEASRESAVVIMNHINLVEILMDVNQWTNVFAGLVSRALTLDVLSTGVAGNYNGALQVMTAEFQVPSPLVPTRENYFVRYCKHHTDGTWAVVDVSLDNLRPSSVSHGRRRPSGCLIQELPNGYSKVTWIEHVEVDDRGVHNIYRPLVNSGLAFGAKRWVATLDRQCERLAS

SEQ ID NO: 26 - protein, 233 aa, Capsicum annuum
IDADKPIIIELAVAAMEELIRMAQTGEPLWIKTLDNSSETLSEEEYFRTFPQGIGPKPLGLTSEASRESAVVIMNHINLVEILMDVNQWTSVFAGLVSRSLTLEVLSTGVAGNYNGALQVMTAEFQVPSPLVPTRENYFVRYCKHHADGTWAVVDVSLDHLRPTAVSRDRRRPSGCLIQELPNGYSKVTWIEHVEVDDRSAHNIYRPLVNSGLAFGAKRWVATLDRQCERLAS

SEQ ID NO: 27 - protein, 233 aa, Cucumis melo
TEADKPMIIELAVAAMEELTRMAQMGEPLWMTTLDGSTHMLNEDEYLRTFPRGIGPKPSGFKCEASRESAVVIMNHINLVEILMDVNQWSTLFSGIVSRAMTLEVLSTGVAGNYNGALQVMTSEFQVPSPLVPTRESYFVRYCKQHGDGTWAVVDVSLDDLRPTPGVRCRRRPSGCLIQEMPNGYSKVTWVEHVEVDDRGVHNLYKQLVSSGQAFGAKRWVTTLDRQCERLAS

SEQ ID NO: 28 - protein, 233 aa, Cucumis sativus
TEADKPMIIELAVAAMEELTRMAQMGEPLWMTTLDGSTHMLNEDEYLRTFPRGIGPKPSGFKCEASRESAVVIMNHINLVEILMDVNQWSTLFSGIVSRAMTLEVLSTGVAGNYNGALQVMTSEFQVPSPLVPTRESYYVRYCKQHGDGTWVVVDVSLDDLRPTPGVRCRRRPSGCLIQEMPNGYSKVTWVEHVEVDDRGVHNLYKQLVSSGQAFGAKRWVTTLDRQCERLAS

SEQ ID NO: 29 - protein, 232 aa, Gossypium hirsutum
TEADKPMIVELAVAAMEELIRMAQSGEPLWVPGDNSTDVLNEDEYLRTFPRGIGPKPLGLRSEASRESAVVIMNHVNLVEILMDVNQWSSVFCGIVSRAMTLEVLSTGVAGNYNGALQVMTAEFQVPSPLVPTRENYFARYCKQHIDGTWAVVDVSLDNLRPNPMSKCRRRPSGCLIQELPNGYSKVIWVEHVEVDDRAVHNIYRPVVNSGLAFGAKRWVATLDRQCERLAS

SEQ ID NO: 30 - protein, 233 aa, Nicotiana tabacum
TDADKPIIIELAVAAMEELIRMAQTGEPLWILSPDNSTETLCVEEYMRTFPRGIGPQPLGLKSEASRESAVVIMNHINLVEILMDVNQWTSVFAGLVSRAVTLEVLSTGVAGNYNGALQVMTAEFQVPSPLVPTRENYFVRYCKHHADGTWAVVDVSLDNLRPTSTSRCRRRPSGCLIQELPNGYSKVTWIEHIEVDDRAVHNIYRPLVNSGLAFGAKRWVATLDRQCERLAS

SEQ ID NO: 31 - protein, 61 aa, synthetic construct
  VARIANT 1: note = K or Q
  VARIANT 2: note = P or S
  VARIANT 3: note = L or I or S
  VARIANT 5: note = L or M or F
  VARIANT 6: note = K or R or I or T
  VARIANT 4: note = S or T or C
  VARIANT 12: note = E or Q
  VARIANT 13: note = S or T or L
  VARIANT 14: note = N or A or S
  VARIANT 18: note = I or M
  VARIANT 19: note = N or D
  VARIANT 20: note = Y or H
  VARIANT 21: note = L or T or I or V
  VARIANT 22: note = H or N or S or T
  VARIANT 30: note = V or T
  VARIANT 34: note = T or S
  VARIANT 31: note = S or N or T
  VARIANT 35: note = N or T or S
  VARIANT 36: note = F or I or M or V or L
  VARIANT 37: note = T or C or A or S
  VARIANT 38: note = G or S
  VARIANT 39: note = I or L
  VARIANT 42: note = K or R
  VARIANT 43: note = S or A
  VARIANT 44: note = T or M or L or V or A
  VARIANT 45: note = L or T
  VARIANT 47: note = E or D
  VARIANT 48: note = V or I
  VARIANT 58: note = Y or H
XXXGXXXEASRXXXVVIXXXXXLVEILMDXXQWXXXFXXXVSXXXXLXXLSTGVAGNXNGA

SEQ ID NO: 32 - DNA, 5206 bp, Salvia sclarea
  source 1..5206: mol_type = genomic DNA
ttgtatggagagtgagaggggtaagaaatttaaaaaagaaaaagagagaattaagtgggtttcaccatacaggcagaggaaatttaaacatcagataccaaccccaagggccttgcaataaaaccaccccagccataaatgccatcacaccctctctatacgctctgcaattactccattcctgccacatcttcttcctcacctcttcctccctaattcttcttcttcatcttcttccttcacccacttttaacatttctcgccctacccacccccctactcatgggtttcttttcctttctttccctttcatcgccatacgctaacaattcttcttaaattctattcacaagaaaggcaccatctgcaataaaacctgaaaacccttcattcttggctgcccaaaactgcttttctgcaatcactttaacctcgaaataccagatctctctttcgccaaaccctaattcaggataagggttttcttccatcaaagtaagtccactcactcacacatttacctcctctatgtctatatattcttcgcaacttctatgttagtgcgctctctaaaaccataattctatttctcccaaaaaacataggaaaacaaacaccataaatctcgcctttcttctcacattcttcatattccaatttagctcctttcctttcctttccttacctttttttttttttttttttcattccgttatgtttttatttttattttattttttggacagagagcgaaaagatttgagtcggacaccaccgaagatctcgtgggcgttatatgtaacaacggtttgataaaaaaaaaaagaaaaacgatacagctagagtgtcaaaggccagttctcactgtcaactccttcgctgcaatttcccttctttgtatttcttttcttttctttttccccttttctcgtttttagtcctttggcacgtcacgacagcagagatgaaaagtcctttttgaaatccaaaaaccaagaaacaaaaaagtccatcaaaccttaaaagaaacaacaaaacaaaagtccattgctagtctgttgttacatgtaaccatcccatttgcttttcgctcactctgccagagaatctaccaaaacttcaacgcacgaacttttagaaaacccagcataactttatattaccctatttttgccagaattagagagacgaatagtttctagggtttatatggtgcttcgttccatctccgattgaatgatttcgccggcgactcggaaaactccgatgccccgacccaaagattagtcggtgagtttttagggttttcctttaaaatcgatgtaggattacaagaatttaatctctgtcttttttttttaagaaaataatctgtacatgaattctgatgtgattaagccctggggttgggaaaaagcgaaccaccttttcgattttcctaaatcattaatttccttgtacattcattctcaatgtactaaaatcattaatttctttgtacactcattctcaatgtagatacattagagatctgattaggccatgagctatcgcatgaagttaaatttcagtataattgttcgattctaaatgtgctaataagtagatataaacctgaatttgctatggtatctccttcaccaggaagagtaatgatagatctgtggccttaatcacacttggagtcaaaattgggcatttttaataaaatattctatgcttaaatgagcgcgattgcaaggaatgtctgtatacataagcattaaaattcttaaaaatgcatttctcaaatgttttcgcatttgaatttgagtgacagatttgtacaagggcgggtgaagcagaaggtagtaagatgtttcagccaaatatgtttgatagccaccatcacctgctggatatggcgcacaaaacaccggagaatgagatggacctgattagagacgaggagtacgagagcaaatcagggactgatattatggaggcaccatccggcgatgatcaagatcccaatcaacgcccaaagaagaagagatatcatcgccacacacagcaccaaatccaggaaatggaatcgtaagctcactacttcttctttctttctttcttcctttctttatttttctttgcctcactaaatacttgaacagcttcttcaatgaatgccctcaccccgacgacaagcagaggaaagagctcggccgacgattaggattagaacctttgcaagttaaattttggtttcaaaacaaacgtactcaaatgaaggttcttgtttttttgttttttaactcctcagatttacatatctcttctttccctgaagaagcttaactgtgcaggcccaacacgagcgccacgagaacacccaattgagaaatgaaaacgagaagctgcgagcggagaatatacgctacaaagaggctctcagcaatgccacctgtcccaactgcggaggtccagcggccattggtgagatgtcatttgacgagcagcatctcaggatagaaaatgctcgcttaagggaagaggtaataatggagaattcaatttctccatctccattaattaggtctggattgagcaataattgatgaatcaatgtaaatatgcagattgataggatatctgggatagctgcaaaatatgttgggaaacctatgctttcatatcctcatctatcccccggcgcatcacggtcgcttgatttgggggtggggaatttcgggagtcagacagggattggtggggaagtttatggagctggtgatcttcttaggtcagtgtcaggccctaccgatgctgataagccggtgatcattgagttggccgttgcagcaatggaggagctcatcagaatggctcaaagtggagatcccttgtggatcccaagcaccgaaaatggtgctgagattttgagtgaggaggaatacggtaggaccttcccccgcgggatcggccccaaacctctaggattgaaatctgaggcatcaagggagtcggccgtcgtcatcatgaaccacatcaacctggttgagatattgatggatgtggtacgaatatattcatcttcatctttatcatcatattcatttatatatgtgatggttgattaatttgaacttgctaatttcagaatcagtggtcgaatgtgtttgctagcattgtttcgagatcagtgactttggaggtgttgtctactggtgtggcaggcaactacaacggagctttacaagtggtatgtatatacaagtaattagttgattaattacatattgatatatagctaacagcaatgtggcactttagatgactgctgagttccaagtgccctctcctttggtcccaacgcgcgagaattactttgtgagatactgcaagcaacataccgatgggacttgggcggtggttgatgtttcgctagacaacttgagacctacttccatttccagatgcagacgacggccatctggttgtttgatacaggagctgcctaatggttactctaaggtaatcaatcattgctctctctagctagtagatcgagtggtcattgtttaacatgttaatttgtttggtaggtgacatgggtagaacatgtagaggtagacgatagagccgtgcacagtatctacaagccactggttaattcgggactagcatttggggctaagcgctgggttgcaactctcgacagacagtgcgaacgacttgcgagcgtcatggctaataacatctcagcaggagacgttggaggtttaaattatattcacctcttctcttctcttctcttttctatctcctctcttctcttctcttgttggatatatatatttataagtaactgtatatgtgttgcagtgatatcaactccagaaggtagaaagagcatgctgaagctggcggagaggatggtgatgagtttctgcacgggcgtcggagcttcgactgcgcacacgtggacgacgctgtccggcagcggcgccgatgacgttcgggtgatgaccagaaagagcatggacgatccgggaaggccgcctggcattgtgctcagcgctgctacttccttctggcttcctgttcctcccaaaagagtttttgatttcctgcgcgacgagaactcgagaagcgaggtattcttttgtttttcctttaccctaaatctaaatctataaacctaatccaatctaatgtaattgaatttgttggtacgatgattaaagtgggatattctctccaatggcggcctcgttcaagaaatggcgcacatcgccaacggccgtgatccaggaaattcggtctccctgctccgcgtcaatgtaagattaattgaacagatttgaagggtttaggatttaggttgctattgaaagtaagttgtgaatttgtacgtacagagcgcgaattcgagccagagcaacatgctaatactgcaggagagcagcacggacgcgacaggatcgtacgtgatctacgcgcctgtagatatccacgcgatgaacattgtcctgagcggcggggaccccgactacgtggccctccttccctccggcttcgccatacttcccgacgggcccaccaacgaagcgcccggagtgcccgaggtgggttcggggggatcgttgctcacggtggcctttcaaatactagtggactccgtccccacggccaagctttcattgggctcagtagcaaccgtcaatagcctcatcaaatgcaccgtagagaggatcaaaggcgcagtgctctgcgacaccgcatgacaacaaccccattggaagagcaagcaggatttgtttacgatggtagaaatgtatcaaagggagaagtcaagaacgcacctcgcgtgatccttgcaagggttcgggtattgactctgcctggttaacttgagatcaagtaaacaaaggacctgctttaatactctatgtattatctctctcttttctctttacaaactaattccttttgttttcttcaaacccaatcttgcttctttttaaccaacgacatcttatgttttttttgcgtcttaccttaccctctttcggaaactcctttcattctttaatattatcaaatttaattcttcttctaccaaaattgacttattaaacttttatttactttttacttcgtcttgcgcgcgtatgtatgaacctaatttgatacagagcttcagcttaatccaaaaaaatatgttatc

SEQ ID NO: 33 - DNA, 2178 bp, Salvia sclarea
  source 1..2178: mol_type = genomic DNA
atgtttcagccaaatatgtttgatagccaccatcacctgctggatatggcgcacaaaacaccggagaatgagatggacctgattagagacgaggagtacgagagcaaatcagggactgatattatggaggcaccatccggcgatgatcaagatcccaatcaacgcccaaagaagaagagatatcatcgccacacacagcaccaaatccaggaaatggaatccttcttcaatgaatgccctcaccccgacgacaagcagaggaaagagctcggccgacgattaggattagaacctttgcaagttaaattttggtttcaaaacaaacgtactcaaatgaaggcccaacacgagcgccacgagaacacccaattgagaaatgaaaacgagaagctgcgagcggagaatatacgctacaaagaggctctcagcaatgccacctgtcccaactgcggaggtccagcggccattggtgagatgtcatttgacgagcagcatctcaggatagaaaatgctcgcttaagggaagagattgataggatatctgggatagctgcaaaatatgttgggaaacctatgctttcatatcctcatctatcccccggcgcatcacggtcgcttgatttgggggtggggaatttcgggagtcagacagggattggtggggaagtttatggagctggtgatcttcttaggtcagtgtcaggccctaccgatgctgataagccggtgatcattgagttggccgttgcagcaatggaggagctcatcagaatggctcaaagtggagatcccttgtggatcccaagcaccgaaaatggtgctgagattttgagtgaggaggaatacggtaggaccttcccccgcgggatcggccccaaacctctaggattgaaatctgaggcatcaagggagtcggccgtcgtcatcatgaaccacatcaacctggttgagatattgatggatgtgaatcagtggtcgaatgtgtttgctagcattgtttcgagatcagtgactttggaggtgttgtctactggtgtggcaggcaactacaacggagctttacaagtgatgactgctgagttccaagtgccctctcctttggtcccaacgcgcgagaattactttgtgagatactgcaagcaacataccgatgggacttgggcggtggttgatgtttcgctagacaacttgagacctacttccatttccagatgcagacgacggccatctggttgtttgatacaggagctgcctaatggttactctaaggtgacatgggtagaacatgtagaggtagacgatagagccgtgcacagtatctacaagccactggttaattcgggactagcatttggggctaagcgctgggttgcaactctcgacagacagtgcgaacgacttgcgagcgtcatggctaataacatctcagcaggagacgttggagtgatatcaactccagaaggtagaaagagcatgctgaagctggcggagaggatggtgatgagtttctgcacgggcgtcggagcttcgactgcgcacacgtggacgacgctgtccggcagcggcgccgatgacgttcgggtgatgaccagaaagagcatggacgatccgggaaggccgcctggcattgtgctcagcgctgctacttccttctggcttcctgttcctcccaaaagagtttttgatttcctgcgcgacgagaactcgagaagcgagtgggatattctctccaatggcggcctcgttcaagaaatggcgcacatcgccaacggccgtgatccaggaaattcggtctccctgctccgcgtcaatagcgcgaattcgagccagagcaacatgctaatactgcaggagagcagcacggacgcgacaggatcgtacgtgatctacgcgcctgtagatatccacgcgatgaacattgtcctgagcggcggggaccccgactacgtggccctccttccctccggcttcgccatacttcccgacgggcccaccaacgaagcgcccggagtgcccgaggtgggttcggggggatcgttgctcacggtggcctttcaaatactagtggactccgtccccacggccaagctttcattgggctcagtagcaaccgtcaatagcctcatcaaatgcaccgtagagaggatcaaaggcgcagtgctctgcgacaccgcatga

SEQ ID NO: 34 - DNA, 5206 bp, Salvia sclarea
  source 1..5206: mol_type = genomic DNA
ttgtatggagagtgagaggggtaagaaatttaaaaaagaaaaagagagaattaagtgggtttcaccatacaggcagaggaaatttaaacatcagataccaaccccaagggccttgcaataaaaccaccccagccataaatgccatcacaccctctctatacgctctgcaattactccattcctgccacatcttcttcctcacctcttcctccctaattcttcttcttcatcttcttccttcacccacttttaacatttctcgccctacccacccccctactcatgggtttcttttcctttctttccctttcatcgccatacgctaacaattcttcttaaattctattcacaagaaaggcaccatctgcaataaaacctgaaaacccttcattcttggctgcccaaaactgcttttctgcaatcactttaacctcgaaataccagatctctctttcgccaaaccctaattcaggataagggttttcttccatcaaagtaagtccactcactcacacatttacctcctctatgtctatatattcttcgcaacttctatgttagtgcgctctctaaaaccataattctatttctcccaaaaaacataggaaaacaaacaccataaatctcgcctttcttctcacattcttcatattccaatttagctcctttcctttcctttccttacctttttttttttttttttttcattccgttatgtttttatttttattttattttttggacagagagcgaaaagatttgagtcggacaccaccgaagatctcgtgggcgttatatgtaacaacggtttgataaaaaaaaaaagaaaaacgatacagctagagtgtcaaaggccagttctcactgtcaactccttcgctgcaatttcccttctttgtatttcttttcttttctttttccccttttctcgtttttagtcctttggcacgtcacgacagcagagatgaaaagtcctttttgaaatccaaaaaccaagaaacaaaaaagtccatcaaaccttaaaagaaacaacaaaacaaaagtccattgctagtctgttgttacatgtaaccatcccatttgcttttcgctcactctgccagagaatctaccaaaacttcaacgcacgaacttttagaaaacccagcataactttatattaccctatttttgccagaattagagagacgaatagtttctagggtttatatggtgcttcgttccatctccgattgaatgatttcgccggcgactcggaaaactccgatgccccgacccaaagattagtcggtgagtttttagggttttcctttaaaatcgatgtaggattacaagaatttaatctctgtcttttttttttaagaaaataatctgtacatgaattctgatgtgattaagccctggggttgggaaaaagcgaaccaccttttcgattttcctaaatcattaatttccttgtacattcattctcaatgtactaaaatcattaatttctttgtacactcattctcaatgtagatacattagagatctgattaggccatgagctatcgcatgaagttaaatttcagtataattgttcgattctaaatgtgctaataagtagatataaacctgaatttgctatggtatctccttcaccaggaagagtaatgatagatctgtggccttaatcacacttggagtcaaaattgggcatttttaataaaatattctatgcttaaatgagcgcgattgcaaggaatgtctgtatacataagcattaaaattcttaaaaatgcatttctcaaatgttttcgcatttgaatttgagtgacagatttgtacaagggcgggtgaagcagaaggtagtaagatgtttcagccaaatatgtttgatagccaccatcacctgctggatatggcgcacaaaacaccggagaatgagatggacctgattagagacgaggagtacgagagcaaatcagggactgatattatggaggcaccatccggcgatgatcaagatcccaatcaacgcccaaagaagaagagatatcatcgccacacacagcaccaaatccaggaaatggaatcgtaagctcactacttcttctttctttctttcttcctttctttatttttctttgcctcactaaatacttgaacagcttcttcaatgaatgccctcaccccgacgacaagcagaggaaagagctcggccgacgattaggattagaacctttgcaagttaaattttggtttcaaaacaaacgtactcaaatgaaggttcttgtttttttgttttttaactcctcagatttacatatctcttctttccctgaagaagcttaactgtgcaggcccaacacgagcgccacgagaacacccaattgagaaatgaaaacgagaagctgcgagcggagaatatacgctacaaagaggctctcagcaatgccacctgtcccaactgcggaggtccagcggccattggtgagatgtcatttgacgagcagcatctcaggatagaaaatgctcgcttaagggaagaggtaataatggagaattcaatttctccatctccattaattaggtctggattgagcaataattgatgaatcaatgtaaatatgcagattgataggatatctgggatagctgcaaaatatgttgggaaacctatgctttcatatcctcatctatcccccggcgcatcacggtcgcttgatttgggggtggggaatttcgggagtcagacagggattggtggggaagtttatggagctggtgatcttcttaggtcagtgtcaggccctaccgatgctgataagccggtgatcattgagttggccgttgcagcaatggaggagctcatcagaatggctcaaagtggagatcccttgtggatcccaagcaccgaaaatggtgctgagattttgagtgaggaggaatacggtaggaccttcccccgcgggatcggccccaaacctctaggattgaaatctgaggcatcaagggagtcggccgtcgtcatcatgaaccacatcaacctggttgagatattgatggatgtggtacgaatatattcatcttcatctttatcatcatattcatttatatatgtgatggttgattaatttgaacttgctaatttcagaatcagtggtcgaatgtgtttgctagcattgtttcgagatcagtgactttggaggtgttgtctactggtgtgtcaggcaactacaacggagctttacaagtggtatgtatatacaagtaattagttgattaattacatattgatatatagctaacagcaatgtggcactttagatgactgctgagttccaagtgccctctcctttggtcccaacgcgcgagaattactttgtgagatactgcaagcaacataccgatgggacttgggcggtggttgatgtttcgctagacaacttgagacctacttccatttccagatgcagacgacggccatctggttgtttgatacaggagctgcctaatggttactctaaggtaatcaatcattgctctctctagctagtagatcgagtggtcattgtttaacatgttaatttgtttggtaggtgacatgggtagaacatgtagaggtagacgatagagccgtgcacagtatctacaagccactggttaattcgggactagcatttggggctaagcgctgggttgcaactctcgacagacagtgcgaacgacttgcgagcgtcatggctaataacatctcagcaggagacgttggaggtttaaattatattcacctcttctcttctcttctcttttctatctcctctcttctcttctcttgttggatatatatatttataagtaactgtatatgtgttgcagtgatatcaactccagaaggtagaaagagcatgctgaagctggcggagaggatggtgatgagtttctgcacgggcgtcggagcttcgactgcgcacacgtggacgacgctgtccggcagcggcgccgatgacgttcgggtgatgaccagaaagagcatggacgatccgggaaggccgcctggcattgtgctcagcgctgctacttccttctggcttcctgttcctcccaaaagagtttttgatttcctgcgcgacgagaactcgagaagcgaggtattcttttgtttttcctttaccctaaatctaaatctataaacctaatccaatctaatgtaattgaatttgttggtacgatgattaaagtgggatattctctccaatggcggcctcgttcaagaaatggcgcacatcgccaacggccgtgatccaggaaattcggtctccctgctccgcgtcaatgtaagattaattgaacagatttgaagggtttaggatttaggttgctattgaaagtaagttgtgaatttgtacgtacagagcgcgaattcgagccagagcaacatgctaatactgcaggagagcagcacggacgcgacaggatcgtacgtgatctacgcgcctgtagatatccacgcgatgaacattgtcctgagcggcggggaccccgactacgtggccctccttccctccggcttcgccatacttcccgacgggcccaccaacgaagcgcccggagtgcccgaggtgggttcggggggatcgttgctcacggtggcctttcaaatactagtggactccgtccccacggccaagctttcattgggctcagtagcaaccgtcaatagcctcatcaaatgcaccgtagagaggatcaaaggcgcagtgctctgcgacaccgcatgacaacaaccccattggaagagcaagcaggatttgtttacgatggtagaaatgtatcaaagggagaagtcaagaacgcacctcgcgtgatccttgcaagggttcgggtattgactctgcctggttaacttgagatcaagtaaacaaaggacctgctttaatactctatgtattatctctctcttttctctttacaaactaattccttttgttttcttcaaacccaatcttgcttctttttaaccaacgacatcttatgttttttttgcgtcttaccttaccctctttcggaaactcctttcattctttaatattatcaaatttaattcttcttctaccaaaattgacttattaaacttttatttactttttacttcgtcttgcgcgcgtatgtatgaacctaatttgatacagagcttcagcttaatccaaaaaaatatgttatc

SEQ ID NO: 35 - DNA, 2178 bp, Salvia sclarea
  source 1..2178: mol_type = genomic DNA
atgtttcagccaaatatgtttgatagccaccatcacctgctggatatggcgcacaaaacaccggagaatgagatggacctgattagagacgaggagtacgagagcaaatcagggactgatattatggaggcaccatccggcgatgatcaagatcccaatcaacgcccaaagaagaagagatatcatcgccacacacagcaccaaatccaggaaatggaatccttcttcaatgaatgccctcaccccgacgacaagcagaggaaagagctcggccgacgattaggattagaacctttgcaagttaaattttggtttcaaaacaaacgtactcaaatgaaggcccaacacgagcgccacgagaacacccaattgagaaatgaaaacgagaagctgcgagcggagaatatacgctacaaagaggctctcagcaatgccacctgtcccaactgcggaggtccagcggccattggtgagatgtcatttgacgagcagcatctcaggatagaaaatgctcgcttaagggaagagattgataggatatctgggatagctgcaaaatatgttgggaaacctatgctttcatatcctcatctatcccccggcgcatcacggtcgcttgatttgggggtggggaatttcgggagtcagacagggattggtggggaagtttatggagctggtgatcttcttaggtcagtgtcaggccctaccgatgctgataagccggtgatcattgagttggccgttgcagcaatggaggagctcatcagaatggctcaaagtggagatcccttgtggatcccaagcaccgaaaatggtgctgagattttgagtgaggaggaatacggtaggaccttcccccgcgggatcggccccaaacctctaggattgaaatctgaggcatcaagggagtcggccgtcgtcatcatgaaccacatcaacctggttgagatattgatggatgtgaatcagtggtcgaatgtgtttgctagcattgtttcgagatcagtgactttggaggtgttgtctactggtgtgtcaggcaactacaacggagctttacaagtgatgactgctgagttccaagtgccctctcctttggtcccaacgcgcgagaattactttgtgagatactgcaagcaacataccgatgggacttgggcggtggttgatgtttcgctagacaacttgagacctacttccatttccagatgcagacgacggccatctggttgtttgatacaggagctgcctaatggttactctaaggtgacatgggtagaacatgtagaggtagacgatagagccgtgcacagtatctacaagccactggttaattcgggactagcatttggggctaagcgctgggttgcaactctcgacagacagtgcgaacgacttgcgagcgtcatggctaataacatctcagcaggagacgttggagtgatatcaactccagaaggtagaaagagcatgctgaagctggcggagaggatggtgatgagtttctgcacgggcgtcggagcttcgactgcgcacacgtggacgacgctgtccggcagcggcgccgatgacgttcgggtgatgaccagaaagagcatggacgatccgggaaggccgcctggcattgtgctcagcgctgctacttccttctggcttcctgttcctcccaaaagagtttttgatttcctgcgcgacgagaactcgagaagcgagtgggatattctctccaatggcggcctcgttcaagaaatggcgcacatcgccaacggccgtgatccaggaaattcggtctccctgctccgcgtcaatagcgcgaattcgagccagagcaacatgctaatactgcaggagagcagcacggacgcgacaggatcgtacgtgatctacgcgcctgtagatatccacgcgatgaacattgtcctgagcggcggggaccccgactacgtggccctccttccctccggcttcgccatacttcccgacgggcccaccaacgaagcgcccggagtgcccgaggtgggttcggggggatcgttgctcacggtggcctttcaaatactagtggactccgtccccacggccaagctttcattgggctcagtagcaaccgtcaatagcctcatcaaatgcaccgtagagaggatcaaaggcgcagtgctctgcgacaccgcatga

SEQ ID NO: 36 - protein, 725 aa, Salvia sclarea
MFQPNMFDSHHHLLDMAHKTPENEMDLIRDEEYESKSGTDIMEAPSGDDQDPNQRPKKKRYHRHTQHQIQEMESFFNECPHPDDKQRKELGRRLGLEPLQVKFWFQNKRTQMKAQHERHENTQLRNENEKLRAENIRYKEALSNATCPNCGGPAAIGEMSFDEQHLRIENARLREEIDRISGIAAKYVGKPMLSYPHLSPGASRSLDLGVGNFGSQTGIGGEVYGAGDLLRSVSGPTDADKPVIIELAVAAMEELIRMAQSGDPLWIPSTENGAEILSEEEYGRTFPRGIGPKPLGLKSEASRESAVVIMNHINLVEILMDVNQWSNVFASIVSRSVTLEVLSTGVSGNYNGALQVMTAEFQVPSPLVPTRENYFVRYCKQHTDGTWAVVDVSLDNLRPTSISRCRRRPSGCLIQELPNGYSKVTWVEHVEVDDRAVHSIYKPLVNSGLAFGAKRWVATLDRQCERLASVMANNISAGDVGVISTPEGRKSMLKLAERMVMSFCTGVGASTAHTWTTLSGSGADDVRVMTRKSMDDPGRPPGIVLSAATSFWLPVPPKRVFDFLRDENSRSEWDILSNGGLVQEMAHIANGRDPGNSVSLLRVNSANSSQSNMLILQESSTDATGSYVIYAPVDIHAMNIVLSGGDPDYVALLPSGFAILPDGPTNEAPGVPEVGSGGSLLTVAFQILVDSVPTAKLSLGSVATVNSLIKCTVERIKGAVLCDTA

SEQ ID NO: 37 - protein, 233 aa, Salvia sclarea
TDADKPVIIELAVAAMEELIRMAQSGDPLWIPSTENGAEILSEEEYGRTFPRGIGPKPLGLKSEASRESAVVIMNHINLVEILMDVNQWSNVFASIVSRSVTLEVLSTGVSGNYNGALQVMTAEFQVPSPLVPTRENYFVRYCKQHTDGTWAVVDVSLDNLRPTSISRCRRRPSGCLIQELPNGYSKVTWVEHVEVDDRAVHSIYKPLVNSGLAFGAKRWVATLDRQCERLAS

SEQ ID NO: 38 - protein, 724 aa, salvia rosmarinus
MFQPNMFDSHHHLLDMSHKTPENDMDLIRDEYESKSGTDIMEAPSGDDQDPNQRPKKKRYHRHTQHQIQEMESFFNECPHPDDKQRKELGRRLALEPLQVKFWFQNKRTQMKAQHERHENTQLRNENEKLRAENIRYKEALSNATCPNCGGPAAIGEMSFDEQHLRIENARLREEIDRISGIAAKYVGKPMLSYPYLSPGASRSLDLGVGNFGGQTGIAGEVYGAADLLRSVSGPTDADKPVIIELAVAAMEELIRMAQSGEPLWMPSTENAAELLSEEEYGRIFPRGIGPKPLGLKSEASRESAVVIMNHIKLVEILMDVNQWSSVFASIVSRSVTLEVLSTGVAGNYNGALQVMTAEFQVPSPLVPTRENYFVRYCKQHTDGTWAVVDVSLDNLRPTSISRCRRRPSGCLIQELPNGYSKVTWVEHVEVDDRAVHSIYKPLVNTGLAFGAKRWVATLDRQCERLASVMANNISAGDVGVISSPEGRKSMLKLAERMVMSFCTGVGASTAHTWTTLSGSGADDVRVMTRKSMDDPGRPPGIVLSAATSFWLPVPPTRVFDFLRDENSRSEWDILSNGGLVQEMAHIANGRDPGNSVSLLRVNSANSSQSNMLILQESSTDSTGSYVIYAPVDIHAMNVVLSGGDPDYVALLPSGFAILPDGPNNEAGGIPEVGSGGSLLTVAFQILVDSVPTAKLSLGSVATVNSLIKCTVERIKGAVLCDTA

SEQ ID NO: 39 - protein, 725 aa, Salvia officinalis
MFQPNMFDSHHHLLDMAHKTPENEMDLIRDDEYESKSGTDIMEAPSGDDQDPNQRPKKKRYHRHTQHQIQEMESFFNECPHPDDKQRKELGRRLGLEPLQVKFWFQNKRTQMKAQHERHENTQLRNENEKLRAENIRYKEALSNATCPNCGGPAAIGEMSFDEQHLRIENARLRDEIDRISGIAAKYVGKPMLSYPHLSPGASRSLDLGVGNFGGQTGIGGEVYGASDLLRSVSGPTDADKPVIIELAVAAMEELIRMAQSGEPLWIPSTEMGAELLSEEEYGRTFPRGIGPKPLGLKSEASRESAVVIMNHINLVEILMDVNQWSSVFASIVSRSVTLEVLSTGVAGNYNGALQVMTAEFQVPSPLVPTRENYFVRYCKQHTDGTWAVVDVSLDNLRPTSISRCRRRPSGCLIQELPNGYSKVTWIEHVEVDDRAVHSIYKPLVNSGLAFGAKRWVAILDRQCERLASVMANNISAGDVGVISSPEGRKSMLKLAERMVMSFCTGVGASTAHTWTTLSGSGADDVRVMTRKSMDDPGRPPGIVLSAATSFWLPVPPKRVFDFLRDENSRSEWDILSNGGLVQEMAHIANGRDPGNSVSLLRVNSANSSQSNMLILQESSTDATGSYVIYAPVDIHAMNVVLSGGDPDYVALLPSGFAILPDGPSNEAGGIPEVGSGGSLLTVAFQILVDSVPTAKLSLGSVATVNSLIKCTVERIKGAVLCETA

SEQ ID NO: 40 - protein, 233 aa, salvia rosmarinus
TDADKPVIIELAVAAMEELIRMAQSGEPLWMPSTENAAELLSEEEYGRIFPRGIGPKPLGLKSEASRESAVVIMNHIKLVEILMDVNQWSSVFASIVSRSVTLEVLSTGVAGNYNGALQVMTAEFQVPSPLVPTRENYFVRYCKQHTDGTWAVVDVSLDNLRPTSISRCRRRPSGCLIQELPNGYSKVTWVEHVEVDDRAVHSIYKPLVNTGLAFGAKRWVATLDRQCERLAS

SEQ ID NO: 41 - protein, 233 aa, Salvia officinalis
TDADKPVIIELAVAAMEELIRMAQSGEPLWIPSTEMGAELLSEEEYGRTFPRGIGPKPLGLKSEASRESAVVIMNHINLVEILMDVNQWSSVFASIVSRSVTLEVLSTGVAGNYNGALQVMTAEFQVPSPLVPTRENYFVRYCKQHTDGTWAVVDVSLDNLRPTSISRCRRRPSGCLIQELPNGYSKVTWIEHVEVDDRAVHSIYKPLVNSGLAFGAKRWVAILDRQCERLAS

SEQ ID NO: 42 - DNA, 26 bp, synthetic construct
  source 1..26: mol_type = other DNA
tgagatggacctgattagagacgagg

SEQ ID NO: 43 - DNA, 23 bp, synthetic construct
  source 1..23: mol_type = other DNA
ctggatatggcgcacaaaacacc

SEQ ID NO: 44 - DNA, 25 bp, synthetic construct
  source 1..25: mol_type = other DNA
gtgcatttgatgaggctattgacgg

SEQ ID NO: 45 - DNA, 25 bp, synthetic construct
  source 1..25: mol_type = other DNA
tagtatttgaaaggccaccgtgagc

SEQ ID NO: 46 - DNA, 5206 bp, Salvia sclarea
  source 1..5206: mol_type = genomic DNA
ttgtatggagagtgagaggggtaagaaatttaaaaaagaaaaagagagaattaagtgggtttcaccatacaggcagaggaaatttaaacatcagataccaaccccaagggccttgcaataaaaccaccccagccataaatgccatcacaccctctctatacgctctgcaattactccattcctgccacatcttcttcctcacctcttcctccctaattcttcttcttcatcttcttccttcacccacttttaacatttctcgccctacccacccccctactcatgggtttcttttcctttctttccctttcatcgccatacgctaacaattcttcttaaattctattcacaagaaaggcaccatctgcaataaaacctgaaaacccttcattcttggctgcccaaaactgcttttctgcaatcactttaacctcgaaataccagatctctctttcgccaaaccctaattcaggataagggttttcttccatcaaagtaagtccactcactcacacatttacctcctctatgtctatatattcttcgcaacttctatgttagtgcgctctctaaaaccataattctatttctcccaaaaaacataggaaaacaaacaccataaatctcgcctttcttctcacattcttcatattccaatttagctcctttcctttcctttccttacctttttttttttttttttttcattccgttatgtttttatttttattttattttttggacagagagcgaaaagatttgagtcggacaccaccgaagatctcgtgggcgttatatgtaacaacggtttgataaaaaaaaaaagaaaaacgatacagctagagtgtcaaaggccagttctcactgtcaactccttcgctgcaatttcccttctttgtatttcttttcttttctttttccccttttctcgtttttagtcctttggcacgtcacgacagcagagatgaaaagtcctttttgaaatccaaaaaccaagaaacaaaaaagtccatcaaaccttaaaagaaacaacaaaacaaaagtccattgctagtctgttgttacatgtaaccatcccatttgcttttcgctcactctgccagagaatctaccaaaacttcaacgcacgaacttttagaaaacccagcataactttatattaccctatttttgccagaattagagagacgaatagtttctagggtttatatggtgcttcgttccatctccgattgaatgatttcgccggcgactcggaaaactccgatgccccgacccaaagattagtcggtgagtttttagggttttcctttaaaatcgatgtaggattacaagaatttaatctctgtcttttttttttaagaaaataatctgtacatgaattctgatgtgattaagccctggggttgggaaaaagcgaaccaccttttcgattttcctaaatcattaatttccttgtacattcattctcaatgtactaaaatcattaatttctttgtacactcattctcaatgtagatacattagagatctgattaggccatgagctatcgcatgaagttaaatttcagtataattgttcgattctaaatgtgctaataagtagatataaacctgaatttgctatggtatctccttcaccaggaagagtaatgatagatctgtggccttaatcacacttggagtcaaaattgggcatttttaataaaatattctatgcttaaatgagcgcgattgcaaggaatgtctgtatacataagcattaaaattcttaaaaatgcatttctcaaatgttttcgcatttgaatttgagtgacagatttgtacaagggcgggtgaagcagaaggtagtaagatgtttcagccaaatatgtttgatagccaccatcacctgctggatatggcgcacaaaacaccggagaatgagatggacctgattagagacgaggagtacgagagcaaatcagggactgatattatggaggcaccatccggcgatgatcaagatcccaatcaacgcccaaagaagaagagatatcatcgccacacacagcaccaaatccaggaaatggaatcgtaagctcactacttcttctttctttctttcttcctttctttatttttctttgcctcactaaatacttgaacagcttcttcaatgaatgccctcaccccgacgacaagcagaggaaagagctcggccgacgattaggattagaacctttgcaagttaaattttggtttcaaaacaaacgtactcaaatgaaggttcttgtttttttgttttttaactcctcagatttacatatctcttctttccctgaagaagcttaactgtgcaggcccaacacgagcgccacgagaacacccaattgagaaatgaaaacgagaagctgcgagcggagaatatacgctacaaagaggctctcagcaatgccacctgtcccaactgcggaggtccagcggccattggtgagatgtcatttgacgagcagcatctcaggatagaaaatgctcgcttaagggaagaggtaataatggagaattcaatttctccatctccattaattaggtctggattgagcaataattgatgaatcaatgtaaatatgcagattgataggatatctgggatagctgcaaaatatgttgggaaacctatgctttcatatcctcatctatcccccggcgcatcacggtcgcttgatttgggggtggggaatttcgggagtcagacagggattggtggggaagtttatggagctggtgatcttcttaggtcagtgtcaggccctaccgatgctgataagccggtgatcattgagttggccgttgcagcaatggaggagctcatcagaatggctcaaagtggagatcccttgtggatcccaagcaccgaaaatggtgctgagattttgagtgaggaggaatacggtaggaccttcccccgcgggatcggccccaaacctctaggattgaaatctgaggcatcaagggagtcggccgtcgtcatcatgaaccacatcaacctggttgagataatgatggatgtggtacgaatatattcatcttcatctttatcatcatattcatttatatatgtgatggttgattaatttgaacttgctaatttcagaatcagtggtcgaatgtgtttgctagcattgtttcgagatcagtgactttggaggtgttgtctactggtgtgtcaggcaactacaacggagctttacaagtggtatgtatatacaagtaattagttgattaattacatattgatatatagctaacagcaatgtggcactttagatgactgctgagttccaagtgccctctcctttggtcccaacgcgcgagaattactttgtgagatactgcaagcaacataccgatgggacttgggcggtggttgatgtttcgctagacaacttgagacctacttccatttccagatgcagacgacggccatctggttgtttgatacaggagctgcctaatggttactctaaggtaatcaatcattgctctctctagctagtagatcgagtggtcattgtttaacatgttaatttgtttggtaggtgacatgggtagaacatgtagaggtagacgatagagccgtgcacagtatctacaagccactggttaattcgggactagcatttggggctaagcgctgggttgcaactctcgacagacagtgcgaacgacttgcgagcgtcatggctaataacatctcagcaggagacgttggaggtttaaattatattcacctcttctcttctcttctcttttctatctcctctcttctcttctcttgttggatatatatatttataagtaactgtatatgtgttgcagtgatatcaactccagaaggtagaaagagcatgctgaagctggcggagaggatggtgatgagtttctgcacgggcgtcggagcttcgactgcgcacacgtggacgacgctgtccggcagcggcgccgatgacgttcgggtgatgaccagaaagagcatggacgatccgggaaggccgcctggcattgtgctcagcgctgctacttccttctggcttcctgttcctcccaaaagagtttttgatttcctgcgcgacgagaactcgagaagcgaggtattcttttgtttttcctttaccctaaatctaaatctataaacctaatccaatctaatgtaattgaatttgttggtacgatgattaaagtgggatattctctccaatggcggcctcgttcaagaaatggcgcacatcgccaacggccgtgatccaggaaattcggtctccctgctccgcgtcaatgtaagattaattgaacagatttgaagggtttaggatttaggttgctattgaaagtaagttgtgaatttgtacgtacagagcgcgaattcgagccagagcaacatgctaatactgcaggagagcagcacggacgcgacaggatcgtacgtgatctacgcgcctgtagatatccacgcgatgaacattgtcctgagcggcggggaccccgactacgtggccctccttccctccggcttcgccatacttcccgacgggcccaccaacgaagcgcccggagtgcccgaggtgggttcggggggatcgttgctcacggtggcctttcaaatactagtggactccgtccccacggccaagctttcattgggctcagtagcaaccgtcaatagcctcatcaaatgcaccgtagagaggatcaaaggcgcagtgctctgcgacaccgcatgacaacaaccccattggaagagcaagcaggatttgtttacgatggtagaaatgtatcaaagggagaagtcaagaacgcacctcgcgtgatccttgcaagggttcgggtattgactctgcctggttaacttgagatcaagtaaacaaaggacctgctttaatactctatgtattatctctctcttttctctttacaaactaattccttttgttttcttcaaacccaatcttgcttctttttaaccaacgacatcttatgttttttttgcgtcttaccttaccctctttcggaaactcctttcattctttaatattatcaaatttaattcttcttctaccaaaattgacttattaaacttttatttactttttacttcgtcttgcgcgcgtatgtatgaacctaatttgatacagagcttcagcttaatccaaaaaaatatgttatc

SEQ ID NO: 47 - DNA, 2178 bp, Salvia sclarea
  source 1..2178: mol_type = genomic DNA
atgtttcagccaaatatgtttgatagccaccatcacctgctggatatggcgcacaaaacaccggagaatgagatggacctgattagagacgaggagtacgagagcaaatcagggactgatattatggaggcaccatccggcgatgatcaagatcccaatcaacgcccaaagaagaagagatatcatcgccacacacagcaccaaatccaggaaatggaatccttcttcaatgaatgccctcaccccgacgacaagcagaggaaagagctcggccgacgattaggattagaacctttgcaagttaaattttggtttcaaaacaaacgtactcaaatgaaggcccaacacgagcgccacgagaacacccaattgagaaatgaaaacgagaagctgcgagcggagaatatacgctacaaagaggctctcagcaatgccacctgtcccaactgcggaggtccagcggccattggtgagatgtcatttgacgagcagcatctcaggatagaaaatgctcgcttaagggaagagattgataggatatctgggatagctgcaaaatatgttgggaaacctatgctttcatatcctcatctatcccccggcgcatcacggtcgcttgatttgggggtggggaatttcgggagtcagacagggattggtggggaagtttatggagctggtgatcttcttaggtcagtgtcaggccctaccgatgctgataagccggtgatcattgagttggccgttgcagcaatggaggagctcatcagaatggctcaaagtggagatcccttgtggatcccaagcaccgaaaatggtgctgagattttgagtgaggaggaatacggtaggaccttcccccgcgggatcggccccaaacctctaggattgaaatctgaggcatcaagggagtcggccgtcgtcatcatgaaccacatcaacctggttgagataatgatggatgtgaatcagtggtcgaatgtgtttgctagcattgtttcgagatcagtgactttggaggtgttgtctactggtgtggcaggcaactacaacggagctttacaagtgatgactgctgagttccaagtgccctctcctttggtcccaacgcgcgagaattactttgtgagatactgcaagcaacataccgatgggacttgggcggtggttgatgtttcgctagacaacttgagacctacttccatttccagatgcagacgacggccatctggttgtttgatacaggagctgcctaatggttactctaaggtgacatgggtagaacatgtagaggtagacgatagagccgtgcacagtatctacaagccactggttaattcgggactagcatttggggctaagcgctgggttgcaactctcgacagacagtgcgaacgacttgcgagcgtcatggctaataacatctcagcaggagacgttggagtgatatcaactccagaaggtagaaagagcatgctgaagctggcggagaggatggtgatgagtttctgcacgggcgtcggagcttcgactgcgcacacgtggacgacgctgtccggcagcggcgccgatgacgttcgggtgatgaccagaaagagcatggacgatccgggaaggccgcctggcattgtgctcagcgctgctacttccttctggcttcctgttcctcccaaaagagtttttgatttcctgcgcgacgagaactcgagaagcgagtgggatattctctccaatggcggcctcgttcaagaaatggcgcacatcgccaacggccgtgatccaggaaattcggtctccctgctccgcgtcaatagcgcgaattcgagccagagcaacatgctaatactgcaggagagcagcacggacgcgacaggatcgtacgtgatctacgcgcctgtagatatccacgcgatgaacattgtcctgagcggcggggaccccgactacgtggccctccttccctccggcttcgccatacttcccgacgggcccaccaacgaagcgcccggagtgcccgaggtgggttcggggggatcgttgctcacggtggcctttcaaatactagtggactccgtccccacggccaagctttcattgggctcagtagcaaccgtcaatagcctcatcaaatgcaccgtagagaggatcaaaggcgcagtgctctgcgacaccgcatga

SEQ ID NO: 48 - protein, 725 aa, Salvia sclarea
MFQPNMFDSHHHLLDMAHKTPENEMDLIRDEEYESKSGTDIMEAPSGDDQDPNQRPKKKRYHRHTQHQIQEMESFFNECPHPDDKQRKELGRRLGLEPLQVKFWFQNKRTQMKAQHERHENTQLRNENEKLRAENIRYKEALSNATCPNCGGPAAIGEMSFDEQHLRIENARLREEIDRISGIAAKYVGKPMLSYPHLSPGASRSLDLGVGNFGSQTGIGGEVYGAGDLLRSVSGPTDADKPVIIELAVAAMEELIRMAQSGDPLWIPSTENGAEILSEEEYGRTFPRGIGPKPLGLKSEASRESAVVIMNHINLVEIMMDVNQWSNVFASIVSRSVTLEVLSTGVAGNYNGALQVMTAEFQVPSPLVPTRENYFVRYCKQHTDGTWAVVDVSLDNLRPTSISRCRRRPSGCLIQELPNGYSKVTWVEHVEVDDRAVHSIYKPLVNSGLAFGAKRWVATLDRQCERLASVMANNISAGDVGVISTPEGRKSMLKLAERMVMSFCTGVGASTAHTWTTLSGSGADDVRVMTRKSMDDPGRPPGIVLSAATSFWLPVPPKRVFDFLRDENSRSEWDILSNGGLVQEMAHIANGRDPGNSVSLLRVNSANSSQSNMLILQESSTDATGSYVIYAPVDIHAMNIVLSGGDPDYVALLPSGFAILPDGPTNEAPGVPEVGSGGSLLTVAFQILVDSVPTAKLSLGSVATVNSLIKCTVERIKGAVLCDTA

SEQ ID NO: 49 - protein, 233 aa, Salvia sclarea
TDADKPVIIELAVAAMEELIRMAQSGDPLWIPSTENGAEILSEEEYGRTFPRGIGPKPLGLKSEASRESAVVIMNHINLVEIMMDVNQWSNVFASIVSRSVTLEVLSTGVAGNYNGALQVMTAEFQVPSPLVPTRENYFVRYCKQHTDGTWAVVDVSLDNLRPTSISRCRRRPSGCLIQELPNGYSKVTWVEHVEVDDRAVHSIYKPLVNSGLAFGAKRWVATLDRQCERLAS

SEQ ID NO: 50 - DNA, 2178 bp, Salvia sclarea
  source 1..2178: mol_type = genomic DNA
atgtttcagccaaatatgtttgatagccaccatcacctgctggatatggcgcacaaaacaccggagaatgagatggacctgattagagacgaggagtacgagagcaaatcagggactgatattatggaggcaccatccggcgatgatcaagatcccaatcaacgcccaaagaagaagagatatcatcgccacacacagcaccaaatccaggaaatggaatccttcttcaatgaatgccctcaccccgacgacaagcagaggaaagagctcggccgacgattaggattagaacctttgcaagttaaattttggtttcaaaacaaacgtactcaaatgaaggcccaacacgagcgccacgagaacacccaattgagaaatgaaaacgagaagctgcgagcggagaatatacgctacaaagaggctctcagcaatgccacctgtcccaactgcggaggtccagcggccattggtgagatgtcatttgacgagcagcatctcaggatagaaaatgctcgcttaagggaagagattgataggatatctgggatagctgcaaaatatgttgggaaacctatgctttcatatcctcatctatcccccggcgcatcacggtcgcttgatttgggggtggggaatttcgggagtcagacagggattggtggggaagtttatggagctggtgatcttcttaggtcagtgtcaggccctaccgatgctgataagccggtgatcattgagttggccgttgcagcaatggaggagctcatcagaatggctcaaagtggagatcccttgtggatcccaagcaccgaaaatggtgctgagattttgagtgaggaggaatacggtaggaccttcccccgcgggatcggccccaaacctctaggattgaaatctgaggcatcaagggagtcggccgtcgtcatcatgaaccacatcaacctggttgagatattgatggatgtgaatcagtggtcgaatgtgtttgctagcattgtttcgtgatcagtgactttggaggtgttgtctactggtgtggcaggcaactacaacggagctttacaagtgatgactgctgagttccaagtgccctctcctttggtcccaacgcgcgagaattactttgtgagatactgcaagcaacataccgatgggacttgggcggtggttgatgtttcgctagacaacttgagacctacttccatttccagatgcagacgacggccatctggttgtttgatacaggagctgcctaatggttactctaaggtgacatgggtagaacatgtagaggtagacgatagagccgtgcacagtatctacaagccactggttaattcgggactagcatttggggctaagcgctgggttgcaactctcgacagacagtgcgaacgacttgcgagcgtcatggctaataacatctcagcaggagacgttggagtgatatcaactccagaaggtagaaagagcatgctgaagctggcggagaggatggtgatgagtttctgcacgggcgtcggagcttcgactgcgcacacgtggacgacgctgtccggcagcggcgccgatgacgttcgggtgatgaccagaaagagcatggacgatccgggaaggccgcctggcattgtgctcagcgctgctacttccttctggcttcctgttcctcccaaaagagtttttgatttcctgcgcgacgagaactcgagaagcgagtgggatattctctccaatggcggcctcgttcaagaaatggcgcacatcgccaacggccgtgatccaggaaattcggtctccctgctccgcgtcaatagcgcgaattcgagccagagcaacatgctaatactgcaggagagcagcacggacgcgacaggatcgtacgtgatctacgcgcctgtagatatccacgcgatgaacattgtcctgagcggcggggaccccgactacgtggccctccttccctccggcttcgccatacttcccgacgggcccaccaacgaagcgcccggagtgcccgaggtgggttcggggggatcgttgctcacggtggcctttcaaatactagtggactccgtccccacggccaagctttcattgggctcagtagcaaccgtcaatagcctcatcaaatgcaccgtagagaggatcaaaggcgcagtgctctgcgacaccgcatga

SEQ ID NO: 51 - DNA, 5206 bp, Salvia sclarea
  source 1..5206: mol_type = genomic DNA
ttgtatggagagtgagaggggtaagaaatttaaaaaagaaaaagagagaattaagtgggtttcaccatacaggcagaggaaatttaaacatcagataccaaccccaagggccttgcaataaaaccaccccagccataaatgccatcacaccctctctatacgctctgcaattactccattcctgccacatcttcttcctcacctcttcctccctaattcttcttcttcatcttcttccttcacccacttttaacatttctcgccctacccacccccctactcatgggtttcttttcctttctttccctttcatcgccatacgctaacaattcttcttaaattctattcacaagaaaggcaccatctgcaataaaacctgaaaacccttcattcttggctgcccaaaactgcttttctgcaatcactttaacctcgaaataccagatctctctttcgccaaaccctaattcaggataagggttttcttccatcaaagtaagtccactcactcacacatttacctcctctatgtctatatattcttcgcaacttctatgttagtgcgctctctaaaaccataattctatttctcccaaaaaacataggaaaacaaacaccataaatctcgcctttcttctcacattcttcatattccaatttagctcctttcctttcctttccttacctttttttttttttttttttcattccgttatgtttttatttttattttattttttggacagagagcgaaaagatttgagtcggacaccaccgaagatctcgtgggcgttatatgtaacaacggtttgataaaaaaaaaaagaaaaacgatacagctagagtgtcaaaggccagttctcactgtcaactccttcgctgcaatttcccttctttgtatttcttttcttttctttttccccttttctcgtttttagtcctttggcacgtcacgacagcagagatgaaaagtcctttttgaaatccaaaaaccaagaaacaaaaaagtccatcaaaccttaaaagaaacaacaaaacaaaagtccattgctagtctgttgttacatgtaaccatcccatttgcttttcgctcactctgccagagaatctaccaaaacttcaacgcacgaacttttagaaaacccagcataactttatattaccctatttttgccagaattagagagacgaatagtttctagggtttatatggtgcttcgttccatctccgattgaatgatttcgccggcgactcggaaaactccgatgccccgacccaaagattagtcggtgagtttttagggttttcctttaaaatcgatgtaggattacaagaatttaatctctgtcttttttttttaagaaaataatctgtacatgaattctgatgtgattaagccctggggttgggaaaaagcgaaccaccttttcgattttcctaaatcattaatttccttgtacattcattctcaatgtactaaaatcattaatttctttgtacactcattctcaatgtagatacattagagatctgattaggccatgagctatcgcatgaagttaaatttcagtataattgttcgattctaaatgtgctaataagtagatataaacctgaatttgctatggtatctccttcaccaggaagagtaatgatagatctgtggccttaatcacacttggagtcaaaattgggcatttttaataaaatattctatgcttaaatgagcgcgattgcaaggaatgtctgtatacataagcattaaaattcttaaaaatgcatttctcaaatgttttcgcatttgaatttgagtgacagatttgtacaagggcgggtgaagcagaaggtagtaagatgtttcagccaaatatgtttgatagccaccatcacctgctggatatggcgcacaaaacaccggagaatgagatggacctgattagagacgaggagtacgagagcaaatcagggactgatattatggaggcaccatccggcgatgatcaagatcccaatcaacgcccaaagaagaagagatatcatcgccacacacagcaccaaatccaggaaatggaatcgtaagctcactacttcttctttctttctttcttcctttctttatttttctttgcctcactaaatacttgaacagcttcttcaatgaatgccctcaccccgacgacaagcagaggaaagagctcggccgacgattaggattagaacctttgcaagttaaattttggtttcaaaacaaacgtactcaaatgaaggttcttgtttttttgttttttaactcctcagatttacatatctcttctttccctgaagaagcttaactgtgcaggcccaacacgagcgccacgagaacacccaattgagaaatgaaaacgagaagctgcgagcggagaatatacgctacaaagaggctctcagcaatgccacctgtcccaactgcggaggtccagcggccattggtgagatgtcatttgacgagcagcatctcaggatagaaaatgctcgcttaagggaagaggtaataatggagaattcaatttctccatctccattaattaggtctggattgagcaataattgatgaatcaatgtaaatatgcagattgataggatatctgggatagctgcaaaatatgttgggaaacctatgctttcatatcctcatctatcccccggcgcatcacggtcgcttgatttgggggtggggaatttcgggagtcagacagggattggtggggaagtttatggagctggtgatcttcttaggtcagtgtcaggccctaccgatgctgataagccggtgatcattgagttggccgttgcagcaatggaggagctcatcagaatggctcaaagtggagatcccttgtggatcccaagcaccgaaaatggtgctgagattttgagtgaggaggaatacggtaggaccttcccccgcgggatcggccccaaacctctaggattgaaatctgaggcatcaagggagtcggccgtcgtcatcatgaaccacatcaacctggttgagatattgatggatgtggtacgaatatattcatcttcatctttatcatcatattcatttatatatgtgatggttgattaatttgaacttgctaatttcagaatcagtggtcgaatgtgtttgctagcattgtttcgtgatcagtgactttggaggtgttgtctactggtgtggcaggcaactacaacggagctttacaagtggtatgtatatacaagtaattagttgattaattacatattgatatatagctaacagcaatgtggcactttagatgactgctgagttccaagtgccctctcctttggtcccaacgcgcgagaattactttgtgagatactgcaagcaacataccgatgggacttgggcggtggttgatgtttcgctagacaacttgagacctacttccatttccagatgcagacgacggccatctggttgtttgatacaggagctgcctaatggttactctaaggtaatcaatcattgctctctctagctagtagatcgagtggtcattgtttaacatgttaatttgtttggtaggtgacatgggtagaacatgtagaggtagacgatagagccgtgcacagtatctacaagccactggttaattcgggactagcatttggggctaagcgctgggttgcaactctcgacagacagtgcgaacgacttgcgagcgtcatggctaataacatctcagcaggagacgttggaggtttaaattatattcacctcttctcttctcttctcttttctatctcctctcttctcttctcttgttggatatatatatttataagtaactgtatatgtgttgcagtgatatcaactccagaaggtagaaagagcatgctgaagctggcggagaggatggtgatgagtttctgcacgggcgtcggagcttcgactgcgcacacgtggacgacgctgtccggcagcggcgccgatgacgttcgggtgatgaccagaaagagcatggacgatccgggaaggccgcctggcattgtgctcagcgctgctacttccttctggcttcctgttcctcccaaaagagtttttgatttcctgcgcgacgagaactcgagaagcgaggtattcttttgtttttcctttaccctaaatctaaatctataaacctaatccaatctaatgtaattgaatttgttggtacgatgattaaagtgggatattctctccaatggcggcctcgttcaagaaatggcgcacatcgccaacggccgtgatccaggaaattcggtctccctgctccgcgtcaatgtaagattaattgaacagatttgaagggtttaggatttaggttgctattgaaagtaagttgtgaatttgtacgtacagagcgcgaattcgagccagagcaacatgctaatactgcaggagagcagcacggacgcgacaggatcgtacgtgatctacgcgcctgtagatatccacgcgatgaacattgtcctgagcggcggggaccccgactacgtggccctccttccctccggcttcgccatacttcccgacgggcccaccaacgaagcgcccggagtgcccgaggtgggttcggggggatcgttgctcacggtggcctttcaaatactagtggactccgtccccacggccaagctttcattgggctcagtagcaaccgtcaatagcctcatcaaatgcaccgtagagaggatcaaaggcgcagtgctctgcgacaccgcatgacaacaaccccattggaagagcaagcaggatttgtttacgatggtagaaatgtatcaaagggagaagtcaagaacgcacctcgcgtgatccttgcaagggttcgggtattgactctgcctggttaacttgagatcaagtaaacaaaggacctgctttaatactctatgtattatctctctcttttctctttacaaactaattccttttgttttcttcaaacccaatcttgcttctttttaaccaacgacatcttatgttttttttgcgtcttaccttaccctctttcggaaactcctttcattctttaatattatcaaatttaattcttcttctaccaaaattgacttattaaacttttatttactttttacttcgtcttgcgcgcgtatgtatgaacctaatttgatacagagcttcagcttaatccaaaaaaatatgttatc

SEQ ID NO: 52 - protein, 334 aa, Salvia sclarea
MFQPNMFDSHHHLLDMAHKTPENEMDLIRDEEYESKSGTDIMEAPSGDDQDPNQRPKKKRYHRHTQHQIQEMESFFNECPHPDDKQRKELGRRLGLEPLQVKFWFQNKRTQMKAQHERHENTQLRNENEKLRAENIRYKEALSNATCPNCGGPAAIGEMSFDEQHLRIENARLREEIDRISGIAAKYVGKPMLSYPHLSPGASRSLDLGVGNFGSQTGIGGEVYGAGDLLRSVSGPTDADKPVIIELAVAAMEELIRMAQSGDPLWIPSTENGAEILSEEEYGRTFPRGIGPKPLGLKSEASRESAVVIMNHINLVEILMDVNQWSNVFASIVS

SEQ ID NO: 53 - protein, 7 aa, Salvia sclarea
LVEILMD

SEQ ID NO: 54 - protein, 8 aa, Salvia sclarea
LSTGVAGN

SEQ ID NO: 55 - protein, 234 aa, synthetic construct
  VARIANT 1: note = S or T
  VARIANT 2: note = D or E
  VARIANT 20: note = I or L or V
  VARIANT 23: note = A or G
  VARIANT 26: note = S or T or A
  VARIANT 46: note = E or D
  VARIANT 32: note = M or I or L
  VARIANT 33: note = P or Q
  VARIANT 34: note = S or T
  VARIANT 34: note = E or D
  VARIANT 36: note = N or NOTHING
  VARIANT 37: note = S or G or NOTHING
  VARIANT 38: note = A or G or L or S or NOTHING
  VARIANT 39: note = A or G or V
  VARIANT 41: note = L or I or M or V
  VARIANT 42: note = L or F
  VARIANT 43: note = S or V or C
  VARIANT 44: note = E or D
  VARIANT 45: note = E or D
  VARIANT 35: note = E or D
  VARIANT 48: note = G or A or V
  VARIANT 49: note = R or T
  VARIANT 50: note = I or T
  VARIANT 63: note = K or I or R
  VARIANT 69: note = E or Q
  VARIANT 70: note = S or L or T
  VARIANT 71: note = A or S
  VARIANT 79: note = K or N or L
  VARIANT 87: note = V or T
  VARIANT 88: note = N or T
  VARIANT 92: note = S or N
  VARIANT 93: note = V or M
  VARIANT 95: note = A or S
  VARIANT 101: note = A or S
  VARIANT 102: note = V or M
  VARIANT 104: note = L or T
  VARIANT 115: note = Y or H
  VARIANT 119: note = L or F
  VARIANT 138: note = N or I
  VARIANT 148: note = T or H
  VARIANT 151: note = T or S
  VARIANT 165: note = T or A or S
  VARIANT 166: note = S or N
  VARIANT 169: note = R or K
  VARIANT 178: note = L or V
  VARIANT 192: note = V or I
  VARIANT 197: note = V or I
  VARIANT 201: note = A or T
  VARIANT 208: note = P or A
  VARIANT 212: note = T or A or S
  VARIANT 219: note = K or R
  VARIANT 224: note = T or I
XXADKPVIIELAVAAMEELXRMXGQXGXPLWXXXXXXXXEXXXXXXYXXXFPRGIGPKPLGLXSEASRXXXVVIMNHIXLVEILMDXXQWSXXFXSIVSRXXTXEVLSTGVAGNXNGAXQVMTAEFQVPSPLVPTREXYFVRYCKQHXDGXWAVVDVSLDNLRPXXISXCRRRPSGCXIQELPNGYSKVTWXEHVEXDDRXVHSIYKXLVNXGLAFGAXRWVAXLDRQCERLAS

SEQ ID NO: 56 - protein, 60 aa, Salvia sclarea
PLGLKSEASRESAVVIMNHINLVEILMDVNQWSNVFASIVSRSVTLEVLSTGVAGNYNGA

SEQ ID NO: 57 - protein, 60 aa, Salvia sclarea
PLGLKSEASRESAVVIMNHINLVEILMDVNQWSNVFASIVSRSVTLEVLSTGVSGNYNGA

SEQ ID NO: 58 - protein, 60 aa, Salvia sclarea
PLGLKSEASRESAVVIMNHINLVEIMMDVNQWSNVFASIVSRSVTLEVLSTGVAGNYNGA

SEQ ID NO: 59 - protein, 41 aa, Salvia sclarea
PLGLKSEASRESAVVIMNHINLVEILMDVNQWSNVFASIVS